European Patent Specification EP 4 225 952 B1, published April 9, 2025. Title: COMPOSITIONS, KITS, METHODS FOR DETECTING AND IDENTIFYING PATHOGENS THAT CAUSE RESPIRATORY TRACT INFECTIONS AND USE THEREOF. Applicant: SANSURE BIOTECH INC. The sequence listing filed with the application follows.

SEQUENCE LISTING (25 sequences)

SEQ ID NO: 1 - DNA, 23 bp, synthetic construct
  misc_feature 1..23: note = influenza A forward primer
  source 1..23: mol_type = other DNA
tctcatggaatggctaaagacaa

SEQ ID NO: 2 - DNA, 19 bp, synthetic construct
  misc_feature 1..19: note = influenza A reverse primer
  source 1..19: mol_type = other DNA
agggcattttggacaaagc

SEQ ID NO: 3 - DNA, 22 bp, synthetic construct
  misc_feature 1..22: note = influenza A probe
  source 1..22: mol_type = other DNA
caccgtgcccagtgagcgagga

SEQ ID NO: 4 - DNA, 25 bp, synthetic construct
  misc_feature 1..25: note = influenza B forward primer
  source 1..25: mol_type = other DNA
tcactcttcgagcgttttaatgaag

SEQ ID NO: 5 - DNA, 22 bp, synthetic construct
  misc_feature 1..22: note = influenza B reverse primer
  source 1..22: mol_type = other DNA
taatcggtgctcttgaccaaat

SEQ ID NO: 6 - DNA, 26 bp, synthetic construct
  misc_feature 1..26: note = influenza B probe
  source 1..26: mol_type = other DNA
agccaattcgagcagctgaaactgcg

SEQ ID NO: 7 - DNA, 18 bp, synthetic construct
  misc_feature 1..18: note = rhinovirus forward primer
  source 1..18: mol_type = other DNA
gcccctgaatgcggctaa

SEQ ID NO: 8 - DNA, 23 bp, synthetic construct
  misc_feature 1..23: note = rhinovirus reverse primer
  source 1..23: mol_type = other DNA
gaaacacggacacccaaagtagt

SEQ ID NO: 9 - DNA, 25 bp, synthetic construct
  misc_feature 1..25: note = rhinovirus probe
  source 1..25: mol_type = other DNA
taatgagcaattgcgggatgggacc

SEQ ID NO: 10 - DNA, 29 bp, synthetic construct
  misc_feature 1..29: note = rhinovirus probe
  source 1..29: mol_type = other DNA
ctagtgcatacaatccagtgtgtrgctag

SEQ ID NO: 11 - DNA, 20 bp, synthetic construct
  misc_feature 1..20: note = respiratory adenovirus forward primer
  source 1..20: mol_type = other DNA
ggatccacctcaaaagtcat

SEQ ID NO: 12 - DNA, 19 bp, synthetic construct
  misc_feature 1..19: note = respiratory adenovirus forward primer
  source 1..19: mol_type = other DNA
tgggcggagttggcgtaga

SEQ ID NO: 13 - DNA, 26 bp, synthetic construct
  misc_feature 1..26: note = respiratory adenovirus reverse primer
  source 1..26: mol_type = other DNA
gttaagagtattacccagaaaaagtt

SEQ ID NO: 14 - DNA, 25 bp, synthetic construct
  misc_feature 1..25: note = respiratory adenovirus probe
  source 1..25: mol_type = other DNA
acatgaagttgctggagaaggggat

SEQ ID NO: 15 - DNA, 28 bp, synthetic construct
  misc_feature 1..28: note = respiratory adenovirus probe
  source 1..28: mol_type = other DNA
cccatggacataaagttactggagaagg

SEQ ID NO: 16 - DNA, 22 bp, synthetic construct
  misc_feature 1..22: note = respiratory syncytial virus forward primer
  source 1..22: mol_type = other DNA
agaacaagatggggcaaatatg

SEQ ID NO: 17 - DNA, 27 bp, synthetic construct
  misc_feature 1..27: note = respiratory syncytial virus reverse primer
  source 1..27: mol_type = other DNA
tatgttgatgcttgcaagttcttttat

SEQ ID NO: 18 - DNA, 28 bp, synthetic construct
  misc_feature 1..28: note = respiratory syncytial virus probe
  source 1..28: mol_type = other DNA
cgtgaacaagcttcacgaaggctccaca

SEQ ID NO: 19 - DNA, 18 bp, synthetic construct
  misc_feature 1..18: note = mycoplasma pneumoniae forward primer
  source 1..18: mol_type = other DNA
ccgtttctccaccgggtt

SEQ ID NO: 20 - DNA, 23 bp, synthetic construct
  misc_feature 1..23: note = mycoplasma pneumoniae reverse primer
  source 1..23: mol_type = other DNA
gttttaggcgcggttatatcatc

SEQ ID NO: 21 - DNA, 28 bp, synthetic construct
  misc_feature 1..28: note = mycoplasma pneumoniae probe
  source 1..28: mol_type = other DNA
ccctggattgggaatgggtacaggtatg

SEQ ID NO: 22 - DNA, 19 bp, synthetic construct
  misc_feature 1..19: note = internal standard forward primer
  source 1..19: mol_type = other DNA
ggggagccaaaagggtcat

SEQ ID NO: 23 - DNA, 25 bp, synthetic construct
  misc_feature 1..25: note = internal standard reverse primer
  source 1..25: mol_type = other DNA
ggctgttgtcatacttctcatggtt

SEQ ID NO: 24 - DNA, 25 bp, synthetic construct
  misc_feature 1..25: note = internal standard probe
  source 1..25: mol_type = other DNA
atctctgccccctctgctgatgccc

SEQ ID NO: 25 - DNA, 90 bp, homo sapiens
  source 1..90: mol_type = genomic DNA
ggggagccaaaagggtcatcatctctgccccctctgctgatgcccccatgttcgtcatgggtgtgaaccatgagaagtatgacaacagcc